European Patent Specification EP 3 180 033 B1, published June 7, 2023. Title: Peptid zur Verwendung in der Reduktion von Nebenwirkungen in Form von immunstimulatorischen Reaktionen/Effekten. Applicant: Friedrich-Schiller-Universität Jena. The sequence listing filed with the application follows.

SEQUENCE LISTING (19 sequences)

SEQ ID NO: 1 - protein, 5 aa, künstliche Sequenz
  Spaltsequenz für Caspase-4
LEVDG

SEQ ID NO: 2 - protein, 5 aa, künstliche Sequenz
  Spaltsequenz für KLK
VQQKS

SEQ ID NO: 3 - protein, 5 aa, künstliche Sequenz
  Spaltsequenz für PLAP
PHIYV

SEQ ID NO: 4 - protein, 8 aa, künstliche Sequenz
  Spaltsequenz für Cathepsin-E
GGAFLVLP

SEQ ID NO: 5 - protein, 8 aa, künstliche Sequenz
  Spaltsequenz für Cathepsin-E
ALAFSLAA

SEQ ID NO: 6 - protein, 5 aa, künstliche Sequenz
  Spaltsequenz für CMV-Protease
PSVSA

SEQ ID NO: 7 - protein, 5 aa, künstliche Sequenz
  Spaltsequenz für EBV-Protease
GSASA

SEQ ID NO: 8 - RNA, 21 nt, künstliche Sequenz
  source 1..21: /mol_type="unassigned RNA" /note="Oligonukleotide" /organism="künstliche Sequenz"
ucauauucgacuuugguugcc

SEQ ID NO: 9 - RNA, 19 nt, künstliche Sequenz
  source 1..19: /mol_type="unassigned RNA" /note="Oligonukleotide" /organism="künstliche Sequenz"
ucaaacuccaucaugaucu

SEQ ID NO: 10 - RNA, 19 nt, künstliche Sequenz
  source 1..19: /mol_type="unassigned RNA" /note="Oligonukleotide" /organism="künstliche Sequenz"
uccaucaugaucuucugga

SEQ ID NO: 11 - RNA, 19 nt, künstliche Sequenz
  source 1..19: /mol_type="unassigned RNA" /note="Oligonukleotide" /organism="künstliche Sequenz"
uucauaaacacaguucucc

SEQ ID NO: 12 - RNA, 19 nt, künstliche Sequenz
  source 1..19: /mol_type="unassigned RNA" /note="Oligonukleotide" /organism="künstliche Sequenz"
ucaaauugaggcacugugc

SEQ ID NO: 13 - RNA, 19 nt, künstliche Sequenz
  source 1..19: /mol_type="unassigned RNA" /note="Oligonukleotide" /organism="künstliche Sequenz"
uuucuucagagcaggagca

SEQ ID NO: 14 - RNA, 19 nt, künstliche Sequenz
  source 1..19: /mol_type="unassigned RNA" /note="Oligonukleotide" /organism="künstliche Sequenz"
auacacacccuuugccuca

SEQ ID NO: 15 - RNA, 19 nt, künstliche Sequenz
  source 1..19: /mol_type="unassigned RNA" /note="Oligonukleotide" /organism="künstliche Sequenz"
auuucaggcucauauuccu

SEQ ID NO: 16 - RNA, 19 nt, künstliche Sequenz
  source 1..19: /mol_type="unassigned RNA" /note="Oligonukleotide" /organism="künstliche Sequenz"
cacaauucccacuuugagc

SEQ ID NO: 17 - RNA, 19 nt, künstliche Sequenz
  source 1..19: /mol_type="unassigned RNA" /note="Oligonukleotide" /organism="künstliche Sequenz"
guuacccacaauucccacu

SEQ ID NO: 18 - RNA, 19 nt, künstliche Sequenz
  source 1..19: /mol_type="unassigned RNA" /note="Oligonukleotide" /organism="künstliche Sequenz"
uuucuucucuuugucuggg

SEQ ID NO: 19 - RNA, 19 nt, künstliche Sequenz
  source 1..19: /mol_type="unassigned RNA" /note="Oligonukleotide" /organism="künstliche Sequenz"
uauucuccaaacaaugugc